European Patent Application EP 4 169 364 A1, published April 26, 2023. Title: METHYLOBACTERIUM COMPOSITIONS FOR FUNGAL DISEASE CONTROL. Applicant: NEWLEAF SYMBIOTICS, INC. The sequence listing filed with the application follows.

SEQUENCE LISTING (60 sequences)

SEQ ID NO: 1 - DNA, 1471 bp, Methylobacterium sp.
  source 1..1471: mol_type = genomic DNA
ggtgatccagccgcaggttcccctacggctaccttgttacgacttcaccccagtcgctgaccctaccgtggtcgcctgcctccttgcggttggcgcagcgccgtcgggtaagaccaactcccatggtgtgacgggcggtgtgtacaaggcccgggaacgtattcaccgtggcatgctgatccacgattactagcgattccgccttcatgcactcgagttgcagagtgcaatccgaactgagacggcttttggggatttgctccagatcgctccttcgcctcccactgtcaccgccattgtagcacgtgtgtagcccatcccgtaagggccatgaggacttgacgtcatccacaccttcctcgcggcttatcaccggcagtctccctagagtgcccaactgaatgatggcaactaaggacgtgggttgcgctcgttgcgggacttaacccaacatctcacgacacgagctgacgacagccatgcagcacctgtgtgcgcgccaccgaagtggaccccaaatctctctgggtaacacgccatgtcaaaggatggtaaggttctgcgcgttgcttcgaattaaaccacatgctccaccgcttgtgcgggcccccgtcaattcctttgagttttaatcttgcgaccgtactccccaggcggaatgctcaaagcgttagctgcgctactgcggtgcaagcaccccaacagctggcattcatcgtttacggcgtggactaccagggtatctaatcctgtttgctccccacgctttcgcgcctcagcgtcagtaatggtccagttggccgccttcgccaccggtgttcttgcgaatatctacgaatttcacctctacactcgcagttccaccaacctctaccatactcaagcgtcccagtatcgaaggccattctgtggttgagccacaggctttcacccccgacttaaaacgccgcctacgcgccctttacgcccagtgattccgagcaacgctagcccccttcgtattaccgcggctgctggcacgaagttagccggggcttattcctccggtaccgtcattatcgtcccggataaaagagctttacaaccctaaggccttcatcactcacgcggcatggctggatcaggcttgcgcccattgtccaatattccccactgctgcctcccgtaggagtctgggccgtgtctcagtcccagtgtggctgatcatcctctcagaccagctactgatcgtcgccttggtaggccgttaccccaccaactagctaatcagacgcgggccgatcttccggcagtaaacctttccccaaaagggcgtatccggtattagccctagtttcccagggttattccgaaccagaaggcacgttcccacgcgttactcacccgtccgccgctgaccccgaaaggcccgctcgacttgcatgtgttaagcctgccgccagcgttcgctctgagccaggatcaaactctc

SEQ ID NO: 2 - DNA, 1471 bp, Methylobacterium sp.
  source 1..1471: mol_type = genomic DNA
ggtgatccagccgcaggttcccctacggctaccttgttacgacttcaccccagtcgctgaccctaccgtggtcgcctgcctccttgcggttggcgcagcgccgtcgggtaagaccaactcccatggtgtgacgggcggtgtgtacaaggcccgggaacgtattcaccgtggcatgctgatccacgattactagcgattccgccttcatgcactcgagttgcagagtgcaatccgaactgagacggcttttggggatttgctccagatcgctccttcgcgtcccactgtcaccgccattgtagcacgtgtgtagcccatcccgtaagggccatgaggacttgacgtcatccacaccttcctcgcggcttatcaccggcagtctccctagagtgcccaactgaatgatggcaactaaggacgtgggttgcgctcgttgcgggacttaacccaacatctcacgacacgagctgacgacagccatgcagcacctgtgtgcgcgccaccgaagtggaccccaaatctctctgggtaacacgccatgtcaaaggatggtaaggttctgcgcgttgcttcgaattaaaccacatgctccaccgcttgtgcgggcccccgtcaattcctttgagttttaatcttgcgaccgtactccccaggcggaatgctcaaagcgttagctgcgctactgcggtgcaagcaccccaacagctggcattcatcgtttacggcgtggactaccagggtatctaatcctgtttgctccccacgctttcgcgcctcagcgtcagtaatggtccagttggccgccttcgccaccggtgttcttgcgaatatctacgaatttcacctctacactcgcagttccaccaacctctaccatactcaagcgtcccagtatcgaaggccattctgtggttgagccacaggctttcacccccgacttaaaacgccgcctacgcgccctttacgcccagtgattccgagcaacgctagcccccttcgtattaccgcggctgctggcacgaagttagccggggcttattcctccggtaccgtcattatcgtcccggataaaagagctttacaaccctaaggccttcatcactcacgcggcatggctggatcaggcttgcgcccattgtccaatattccccactgctgcctcccgtaggagtctgggccgtgtctcagtcccagtgtggctgatcatcctctcagaccagctactgatcgtcgccttggtaggccgttaccccaccaactagctaatcagacgcgggccgatcttccggcagtaaacctttccccaaaagggcgtatccggtattagccctagtttcccagggttattccgaaccagaaggcacgttcccacgcgttactcacccgtccgccgctgaccccgaagggcccgctcgacttgcatgtgttaagcctgccgccagcgttcgctctgagccaggatcaaactctc

SEQ ID NO: 3 - DNA, 1472 bp, Methylobacterium sp.
  source 1..1472: mol_type = genomic DNA
gagtttgatcctggctcagagcgaacgctggcggcaggcttaacacatgcaagtcgaacgggcttcttcggaagtcagtggcagacgggtgagtaacacgtgggaacgtgcccttcggttcggaataactcagggaaacttgagctaataccggatacgcccttatggggaaaggtttactgccgaaggatcggcccgcgtctgattagcttgttggtggggtaacggcctaccaaggcgacgatcagtagctggtctgagaggatgatcagccacactgggactgagacacggcccagactcctacgggaggcagcagtggggaatattggacaatgggcgcaagcctgatccagccatgccgcgtgagtgatgaaggccttagggttgtaaagctcttttgtccgggacgataatgacggtaccggaagaataagccccggctaacttcgtgccagcagccgcggtaatacgaagggggctagcgttgctcggaatcactgggcgtaaagggcgcgtaggcggccgattaagtcgggggtgaaagcctgtggctcaaccacagaattgccttcgatactggttggcttgagaccggaagaggacagcggaactgcgagtgtagaggtgaaattcgtagatattcgcaagaacaccagtggcgaaggcggctgtctggtccggttctgacgctgaggcgcgaaagcgtggggagcaaacaggattagataccctggtagtccacgccgtaaacgatgaatgccagccgttggtctgcttgcaggtcagtggcgccgctaacgcattaagcattccgcctggggagtacggtcgcaagattaaaactcaaaggaattgacgggggcccgcacaagcggtggagcatgtggtttaattcgaagcaacgcgcagaaccttaccatcccttgacatggcatgttacctcgagagatcggggatcctcttcggaggcgtgcacacaggtgctgcatggctgtcgtcagctcgtgtcgtgagatgttgggttaagtcccgcaacgagcgcaacccacgtccttagttgccatcattcagttgggcactctagggagactgccggtgataagccgcgaggaaggtgtggatgacgtcaagtcctcatggcccttacgggatgggctacacacgtgctacaatggcggtgacagtgggacgcgaaaccgcgaggttgagcaaatccccaaaagccgtctcagttcggattgcactctgcaactcgggtgcatgaaggcggaatcgctagtaatcgtggatcagcacgccacggtgaatacgttcccgggccttgtacacaccgcccgtcacaccatgggagttggtcttacccgacggcgctgcgccaaccgcaagggggcaggcgaccacggtagggtcagcgactggggtgaagtcgtaacaaggtagccgtaggggaacctgcggctggatcacct

SEQ ID NO: 4 - DNA, 1473 bp, Methylobacterium sp.
  source 1..1473: mol_type = genomic DNA
ggtgatccagccgcaggttcccctacggctaccttgttacgacttcaccccagtcgctgaccctaccgtggtcgcctgcctccttgcggttggcgcagcgccgtcgggtaagaccaactcccatggtgtgacgggcggtgtgtacaaggcccgggaacgtattcaccgtggcgtgctgatccacgattactagcgattccgccttcatgcacccgagttgcagagtgcaatccgaactgagacggtttttggggatttgctccacctcgcggcttcgcgtcccactgtcaccgccattgtagcacgtgtgtagcccatcccgtaagggccatgaggacttgacgtcatccacaccttcctcgcggcttatcaccggcagtctccctagagtgcccaactgaatgatggcaactaaggacgtgggttgcgctcgttgcgggacttaacccaacatctcacgacacgagctgacgacagccatgcagcacctgtgtgcacgcctccgaagaggatccccgatctctcgaggtaacatgccatgtcaagggatggtaaggttctgcgcgttgcttcgaattaaaccacatgctccaccgcttgtgcgggcccccgtcaattcctttgagttttaatcttgcgaccgtactccccaggcggaatgcttaatgcgttagcggcgccactgacctgcaagcaggccaacggctggcattcatcgtttacggcgtggactaccagggtatctaatcctgtttgctccccacgctttcgcgcctcagcgtcagaaccggaccagacagccgccttcgccactggtgttcttgcgaatatctacgaatttcacctctacactcgcagttccgctgtcctcttccggtctcaagccaaccagtatcgaaggcaattctgtggttgagccacaggctttcacccccgacttaatcggccgcctacgcgccctttacgcccagtgattccgagcaacgctagcccccttcgtattaccgcggctgctggcacgaagttagccggggcttattcttccggtaccgtcattatcgtcccggacaaaagagctttacaaccctaaggccttcatcactcacgcggcatggctggatcaggcttgcgcccattgtccaatattccccactgctgcctcccgtaggagtctgggccgtgtctcagtcccagtgtggctgatcatcctctcagaccagctactgatcgtcgccttggtaggccgttaccccaccaacaagctaatcagacgcgggccgatccttcggcagtaaacctttccccaaaagggcgtatccggtattagctcaagtttccctgagttattccgaaccgaagggtacgttcccacgtgttactcacccgtctgccactgacacccgaaggtgcccgttcgacttgcatgtgttaagcctgccgccagcgttcgctctgagccaggatcaaactctc

SEQ ID NO: 5 - DNA, 1484 bp, Methylobacterium sp.
  source 1..1484: mol_type = genomic DNA
ggtgatccagccgcaggttcccctacggctaccttgttacgacttcaccccagtcgctgaccctaccgtggtcgcctgcctccagtcgagcaagctcgatttggttggcgcagcgccgtcgggtaagaccaactcccatggtgtgacgggcggtgtgtacaaggcccgggaacgtattcaccgtggcatgctgatccacgattactagcgattccgccttcatgcacgcgagttgcagcgtgcaatccgaactgagacggcttttggagattggctccgggtcaccccttcgcgtcccactgtcaccgccattgtagcacgtgtgtagcccatcccgtaagggccatgaggacttgacgtcatccacaccttcctcgcggcttatcaccggcagtctccctagagtgcccaaccaaatgatggcaactaaggacgtgggttgcgctcgttgcgggacttaacccaacatctcacgacacgagctgacgacagccatgcagcacctgtgtgcgcgcccccgaaggggacctggaatctctcccagtaacacgccatgtcaaaggatggtaaggttctgcgcgttgcttcgaattaaaccacatgctccaccgcttgtgcgggcccccgtcaattcctttgagttttaatcttgcgaccgtactccccaggcggaatgcttaatgcgttagctgcgctactgcggtgcatgcaccccaacagctagcattcatcgtttacggcgtggactaccagggtatctaatcctgtttgctccccacgctttcgcgcctcagcgtcagtaatggtccagttggccgccttcgccaccggtgttcttgcgaatatctacgaatttcacctctacactcgcagttccaccaacctctaccatactcaagcgtcccagtatcgaaggccattctgtggttgagccacaggctttcacccccgacttaaaacgccgcctacgcgccctttacgcccagtgattccgagcaacgctagcccccttcgtattaccgcggctgctggcacgaagttagccggggcttattcctccggtaccgtcattatcgtcccggagaaaagagctttacaaccctaaggccgtcatcactcacgcggcatggctggatcaggcttgcgcccattgtccaatattccccactgctgcctcccgtaggagtctgggccgtgtctcagtcccagtgtggctgatcatcctctcagaccagctactgatcgtcgccttggtaggccgttaccccaccaacaagctaatcagacgcgggccgatcctccggcagtaaacctttctgccaaagcacgtatccggtattagccctagtttcccagggttatcccagaccggagggcacgttcccacgtgttactcacccgtctgccactcaccttgcggtgcgttcgacttgcatgtgttaagcctgccgccagcgttcgctctgagccaggatcaaactctc

SEQ ID NO: 6 - DNA, 1484 bp, Methylobacterium sp.
  source 1..1484: mol_type = genomic DNA
gagtttgatcctggctcagagcgaacgctggcggcaggcttaacacatgcaagtcgaacgcaccgcaaggtgagtggcagacgggtgagtaacacgtgggaacgtgccctccggtctgggataaccctgggaaactagggctaataccggatacgtgctttggcagaaaggtttactgccggaggatcggcccgcgtctgattagcttgttggtggggtaacggcctaccaaggcgacgatcagtagctggtctgagaggatgatcagccacactgggactgagacacggcccagactcctacgggaggcagcagtggggaatattggacaatgggcgcaagcctgatccagccatgccgcgtgagtgatgacggccttagggttgtaaagctcttttctccgggacgataatgacggtaccggaggaataagccccggctaacttcgtgccagcagccgcggtaatacgaagggggctagcgttgctcggaatcactgggcgtaaagggcgcgtaggcggcgttttaagtcgggggtgaaagcctgtggctcaaccacagaatggccttcgatactgggacgcttgagtatggtagaggttggtggaactgcgagtgtagaggtgaaattcgtagatattcgcaagaacaccggtggcgaaggcggccaactggaccattactgacgctgaggcgcgaaagcgtggggagcaaacaggattagataccctggtagtccacgccgtaaacgatgaatgctagctgttggggtgcatgcaccgcagtagcgcagctaacgcattaagcattccgcctggggagtacggtcgcaagattaaaactcaaaggaattgacgggggcccgcacaagcggtggagcatgtggtttaattcgaagcaacgcgcagaaccttaccatcctttgacatggcgtgttactgggagagattccaggtccccttcgggggcgcgcacacaggtgctgcatggctgtcgtcagctcgtgtcgtgagatgttgggttaagtcccgcaacgagcgcaacccacgtccttagttgccatcatttggttgggcactctagggagactgccggtgataagccgcgaggaaggtgtggatgacgtcaagtcctcatggcccttacgggatgggctacacacgtgctacaatggcggtgacagtgggacgcgaaggggtgacccggagccaatctccaaaagccgtctcagttcggattgcacgctgcaactcgcgtgcatgaaggcggaatcgctagtaatcgtggatcagcatgccacggtgaatacgttcccgggccttgtacacaccgcccgtcacaccatgggagttggtcttacccgacggcgctgcgccaaccaaatcgagcttgctcgactggaggcaggcgaccacggtagggtcagcgactggggtgaagtcgtaacaaggtagccgtaggggaacctgcggctggatcacctc

SEQ ID NO: 7 - DNA, 1472 bp, Methylobacterium sp.
  source 1..1472: mol_type = genomic DNA
gagtttgatcctggctcagagcgaacgctggcggcaggcttaacacatgcaagtcgaacgggcttcttcggaagtcagtggcagacgggtgagtaacacgtgggaacgtgcccttcggttcggaataactcagggaaacttgagctaataccggatacgcccttacggggaaaggtttactgccgaaggatcggcccgcgtctgattagcttgttggtggggtaacggcctaccaaggcgacgatcagtagctggtctgagaggatgatcagccacactgggactgagacacggcccagactcctacgggaggcagcagtggggaatattggacaatgggcgcaagcctgatccagccatgccgcgtgagtgatgaaggccttagggttgtaaagctcttttgtccgggacgataatgacggtaccggaagaataagccccggctaacttcgtgccagcagccgcggtaatacgaagggggctagcgttgctcggaatcactgggcgtaaagggcgcgtaggcggccgattaagtcgggggtgaaagcctgtggctcaaccacagaattgccttcgatactggttggcttgagaccggaagaggacagcggaactgcgagtgtagaggtgaaattcgtagatattcgcaagaacaccagtggcgaaggcggctgtctggtccggttctgacgctgaggcgcgaaagcgtggggagcaaacaggattagataccctggtagtccacgccgtaaacgatgaatgccagccgttggtctgcttgcaggtcagtggcgccgctaacgcattaagcattccgcctggggagtacggtcgcaagattaaaactcaaaggaattgacgggggcccgcacaagcggtggagcatgtggtttaattcgaagcaacgcgcagaaccttaccatcccttgacatggcatgttacctcgagagatcggggatcctcttcggaggcgtgcacacaggtgctgcatggctgtcgtcagctcgtgtcgtgagatgttgggttaagtcccgcaacgagcgcaacccacgtccttagttgccatcattcagttgggcactctagggagactgccggtgataagccgcgaggaaggtgtggatgacgtcaagtcctcatggcccttacgggatgggctacacacgtgctacaatggcggtgacagtgggacgcgaaaccgcgaggttgagcaaatccccaaaagccgtctcagttcggattgcactctgcaactcgggtgcatgaaggcggaatcgctagtaatcgtggatcagcacgccacggtgaatacgttcccgggccttgtacacaccgcccgtcacaccatgggagttggtcttacccgacggcgctgcgccaaccgcaagggggcaggcgaccacggtagggtcagcgactggggtgaagtcgtaacaaggtagccgtaggggaacctgcggctggatcacct

SEQ ID NO: 8 - DNA, 1473 bp, Methylobacterium sp.
  source 1..1473: mol_type = genomic DNA
ggtgatccagccgcaggttcccctacggctaccttgttacgacttcaccccagtcgctgaccctaccgtggtcgcctgctccccttgcgggtcggcgcagcgccgtcgggtaagaccaactcccatggtgtgacgggcggtgtgtacaaggcccgggaacgtattcaccgtggcatgctgatccacgattactagcgattccgccttcatgcactcgagttgcagagtgcaatccgaactgagacggcttttggagatttgcttgccctcgcgggttcgcgtcccactgtcaccgccattgtagcacgtgtgtagcccatcccgtaagggccatgaggacttgacgtcatccacaccttcctcgcggcttatcaccggcagtctccccagagtgcccaactgaatgatggcaactgaggacgtgggttgcgctcgttgcgggacttaacccaacatctcacgacacgagctgacgacagccatgcagcacctgtgtgcgcgctcccgaaggagaccgtggatctctccacgtaacacgccatgtcaaaggatggtaaggttctgcgcgttgcttcgaattaaaccacatgctccaccgcttgtgcgggcccccgtcaattcctttgagttttaatcttgcgaccgtactccccaggcggaatgctcaaagcgttagctgcgccactgagaggcaagccccccaacggctggcattcatcgtttacggcgtggactaccagggtatctaatcctgtttgctccccacgctttcgcgcctcagcgtcagtgtcggaccagttggccgccttcgccaccggtgttcttgcgaatatctacgaatttcacctctacactcgcagttccaccaacctcttccgaactcaagtctcccagtatcgaaggcaattctgtggttgagccacaggctttcacccccgacttaaaagaccgcctacgcgccctttacgcccagtgattccgagcaacgctagcccccttcgtattaccgcggctgctggcacgaagttagccggggcttattcctccggtaccgtcattatcgtcccggataaaagagctttacaaccctaaggccttcatcactcacgcggcatggctggatcaggcttgcgcccattgtccaatattccccactgctgcctcccgtaggagtctgggccgtgtctcagtcccagtgtggctgatcatcctctcagaccagctactgatcgtcgccttggtaggccgttaccccaccaactagctaatcagacgcgggccgatcttccggcagtaaacctttccccaaaagggcgtatccggtattagctcaagtttccctgagttattccgaaccagaaggcacgttcccacgcgttactcacccgtccgccgctgacaccgaagtgcccgctcgacttgcatgtgttaagcctgccgccagcgttcgctctgagccaggatcaaactctc

SEQ ID NO: 9 - DNA, 300 bp, Methylobacterium sp.
  source 1..300: mol_type = genomic DNA
acggtcaccccacggactgggcgagtacctcaccggtgttctatcataacgccgagttagttttcgaccgtcccttatgcgatgtaccaccggtgtcggcagccgatttcgtcccaccgggagctggcgttccggttcagaccaccatcatcggtcacgatgtctggattggacacggggccttcatctcccccggcgtgactataggaaacggcgcgatcgtcggggcccaggcggtcgtcacaagagatgtcccaccctatgcggtagttgctggcgtccccgcgaccgtacgacgat

SEQ ID NO: 10 - DNA, 300 bp, Methylobacterium sp.
  source 1..300: mol_type = genomic DNA
ccaataaaagcgttggccgcctgggcaacccgatccgagcctaagactcaaagcgcaagcgaacacttggtagagacagcccgccgactacggcgttccagcactctccggctttgatcggataggcattggtcaaggtgccggtggtgatgacctcgcccgccgcaagcggcgaattactcggatcagcggccagcacctcgaccaagtgtcggagcgcgaccaaagggccacgttcgaggacgtttgaggcgcgaccagtctcgatagtctcatcgtcgcggcgaagctgcacctcga

SEQ ID NO: 11 - DNA, 300 bp, Methylobacterium sp.
  source 1..300: mol_type = genomic DNA
cgatggcaccgacctgccatgcctctgccgtccgcgccagaatggtaaagaggacgaagggggtaaggatcgtcgctgcagtgttgagcagcgaccagagaagggggccgaacatcggcatcaaacctcgattgccactcggacgcgaagcgcgtcttgaaggagggatggaagcgaaacggccgcagagtaaccgccgacgaaagattgcacccctcatcgagcaggatcggaggtgaaggcaagcgtgggttattggtaagtgcaaaaaatataatggtagcgtcagatctagcgttc

SEQ ID NO: 12 - DNA, 23 bp, synthetic construct
  misc_feature 1..23: note = primer
  source 1..23: mol_type = other DNA
cctcaccggtgttctatcataac

SEQ ID NO: 13 - DNA, 20 bp, synthetic construct
  misc_feature 1..20: note = Primer
  source 1..20: mol_type = other DNA
ccgatgatggtggtctgaac

SEQ ID NO: 14 - DNA, 21 bp, synthetic construct
  misc_feature 1..21: note = Probe
  source 1..21: mol_type = other DNA
cgtcccttatgcgatgtacca

SEQ ID NO: 15 - DNA, 22 bp, synthetic construct
  misc_feature 1..22: note = Primer
  source 1..22: mol_type = other DNA
gatccgagcctaagactcaaag

SEQ ID NO: 16 - DNA, 21 bp, synthetic construct
  misc_feature 1..21: note = Primer
  source 1..21: mol_type = other DNA
gaccaatgcctatccgatcaa

SEQ ID NO: 17 - DNA, 20 bp, synthetic construct
  misc_feature 1..20: note = Probe
  source 1..20: mol_type = other DNA
aacacttggtagagacagcc

SEQ ID NO: 18 - DNA, 21 bp, synthetic construct
  misc_feature 1..21: note = Primer
  source 1..21: mol_type = other DNA
aaggagggatggaagcgaaac

SEQ ID NO: 19 - DNA, 19 bp, synthetic construct
  misc_feature 1..19: note = Primer
  source 1..19: mol_type = other DNA
ataacccacgcttgccttc

SEQ ID NO: 20 - DNA, 21 bp, synthetic construct
  misc_feature 1..21: note = Probe
  source 1..21: mol_type = other DNA
cgcagagtaaccgccgacgaa

SEQ ID NO: 21 - DNA, 300 bp, Methylobacterium sp.
  source 1..300: mol_type = genomic DNA
gcccttctgtcaggcgatattgtataatggcgttgccccaatagaagcagccattcgtgcgagggcagcagcgacgctaggtcgaaagagcatcctaatctcgatcaagatgcgactgagatttctgatgaaaatatctagacacaagcaaagctggtgaaattacaacgatcatggcgacaattgcggccaattcggccggaacttgaaggaacataaaaatgaatattacaaatataccgcaaagcatgtagagttgctacaccaagggtcgggacgtccaaaaaaactcactgagga

SEQ ID NO: 22 - DNA, 300 bp, Methylobacterium sp.
  source 1..300: mol_type = genomic DNA
ggaacataaaaatgaatattacaaatataccgcaaagcatgtagagttgctacaccaagggtcgggacgtccaaaaaaactcactgaggaagtcgactggaagcacgaggcgccccccccaggagcggggcgaccggcaagggggcccgcaattgtcgccatgatcgaccagcttaggtaggatcctctttcgacctaacgaatggctgcttctattggggcaacgccattatacaatatcgcctgaccatctggaacgcggcccggtccaccggcaggttggcgacgacagcgtcggag

SEQ ID NO: 23 - DNA, 300 bp, Methylobacterium sp.
  source 1..300: mol_type = genomic DNA
cggcgtcgaccagccgggcgaactgcttgggcatgctctcccgcgacgccggccacagccgcgtccccgtccctccgcacaggatcatcgggtggatttgaaaggcaaaacgggacatcaggataggccgctcaggcgttggcgctgaggcgcttgatgtcggcgtcgaccatctcggtgatcagcgcctcgaggctggtctcggcctcccagccgaaggtcgccttggccttggcggggttgcccagcagcacctcgacctctgccggccggaacagcgccgggtcgacgatcaggtgg

SEQ ID NO: 24 - DNA, 300 bp, Methylobacterium sp.
  source 1..300: mol_type = genomic DNA
ctggacatgcgcccaccccggccaagtccgaccgcaccggcaaccgctcctgtagtcgtcgtcatcgttctcacccctgaggcggagaccgtccgctaacggggtgtctcaagcaaccgtggggcggaggaacacgcacgtagtcgcgtttcaaggttcgcacgaacgcctcggccatgccgttgctctgcgggctctccagcggcgtcgtttttggcaccaaaccaaggtcgcgggcgaagcggcgcgtgtcgcggggactgtcaggaatttcgtgtgggggcggccatagtggatccg

SEQ ID NO: 25 - DNA, 18 bp, synthetic construct
  misc_feature 1..18: note = Primer
  source 1..18: mol_type = other DNA
cacaagcaaagctggtga

SEQ ID NO: 26 - DNA, 19 bp, synthetic construct
  misc_feature 1..19: note = Primer
  source 1..19: mol_type = other DNA
aagatatgctttgcgggta

SEQ ID NO: 27 - DNA, 18 bp, synthetic construct
  misc_feature 1..18: note = Probe
  source 1..18: mol_type = other DNA
cgatcatggcgacaattg

SEQ ID NO: 28 - DNA, 20 bp, synthetic construct
  misc_feature 1..20: note = Primer
  source 1..20: mol_type = other DNA
caatatcgcctgacagaagg

SEQ ID NO: 29 - DNA, 20 bp, synthetic construct
  misc_feature 1..20: note = Primer
  source 1..20: mol_type = other DNA
cacttcaacaaaggcgatca

SEQ ID NO: 30 - DNA, 14 bp, synthetic construct
  misc_feature 1..14: note = Probe
  source 1..14: mol_type = other DNA
ttggcgacgacagc

SEQ ID NO: 31 - DNA, 19 bp, synthetic construct
  misc_feature 1..19: note = Primer
  source 1..19: mol_type = other DNA
actgcttgggcatgctctc

SEQ ID NO: 32 - DNA, 20 bp, synthetic construct
  misc_feature 1..20: note = Primer
  source 1..20: mol_type = other DNA
cctatcctgatgtcccgttt

SEQ ID NO: 33 - DNA, 20 bp, synthetic construct
  misc_feature 1..20: note = Probe
  source 1..20: mol_type = other DNA
aggatcatcgggtggatttg

SEQ ID NO: 34 - DNA, 18 bp, synthetic construct
  misc_feature 1..18: note = Primer
  source 1..18: mol_type = other DNA
aggaacacgcacgtagtc

SEQ ID NO: 35 - DNA, 18 bp, synthetic construct
  misc_feature 1..18: note = Primer
  source 1..18: mol_type = other DNA
ccacacgaaattcctgac

SEQ ID NO: 36 - DNA, 14 bp, synthetic construct
  misc_feature 1..14: note = Probe
  source 1..14: mol_type = other DNA
tggcaccaaaccaa

SEQ ID NO: 37 - DNA, 300 bp, Methylobacterium sp.
  source 1..300: mol_type = genomic DNA
gcaaaacgacctaatagttctacagcggcatgcgccaagtcagcgcggtgaacagtatacctgggagcaacttgtcctccgaaacccacataaaacaaattactcctggcagtgcccagtccatcaaaatcgaatacaatatttctcgaggaggcatctgtaatagcctgccaaagcaacaaagctatggcgccgttatgactttcattgcttctggtagacataaaataatatgccgatttgtgatcccaaatgtagaatattgccgcatcaattgcgccaagtttatttcggatcgat

SEQ ID NO: 38 - DNA, 300 bp, Methylobacterium sp.
  source 1..300: mol_type = genomic DNA
ggcgccaacggtatgatcgcatgattttcctgcggcatagcttgcgggaatggcgtatttggcgctctcctcaggaatttctaagggcatacgcaggaactctacagcacttttactggtattttgtagtgacagcggaggaggctggtgctcaaggtaatcgtgatgaagtgatccgggccattcggggcgcgtttctagtctttccaatccgcgccctgtaccacgtattacgccggaccggtctgcgccgcgccgccctcttgaccgccctaaatgtctaagagcgtctaacaaagc

SEQ ID NO: 39 - DNA, 300 bp, Methylobacterium sp.
  source 1..300: mol_type = genomic DNA
gacgatatcgctcatcttcactgcattgaagctggtgccgtactgcatagggatgaaaaagtgatgcggatagacggctgacgggaaagcgcctggtcgatcgaagactttgctgacgaggttgtggtagccccggatataggcatcgaaggccgggacgttgatcccatcctttgccttatcttgactggcgtcgtcgcgtgccgtcagaacgggcacgtcgcaggtcatcgaggccagcaccttgcggaacacctgcgttccgccgttgggattatcgacggcgaacgcggtggccgc

SEQ ID NO: 40 - DNA, 21 bp, synthetic construct
  misc_feature 1..21: note = Primer
  source 1..21: mol_type = other DNA
gtcctccgaaacccacataaa

SEQ ID NO: 41 - DNA, 23 bp, synthetic construct
  misc_feature 1..23: note = Primer
  source 1..23: mol_type = other DNA
ctaccagaagcaatgaaagtcat

SEQ ID NO: 42 - DNA, 22 bp, synthetic construct
  misc_feature 1..22: note = Probe
  source 1..22: mol_type = other DNA
tctgtaatagcctgccaaagca

SEQ ID NO: 43 - DNA, 19 bp, synthetic construct
  misc_feature 1..19: note = Primer
  source 1..19: mol_type = other DNA
ggctggtgctcaaggtaat

SEQ ID NO: 44 - DNA, 20 bp, synthetic construct
  misc_feature 1..20: note = Primer
  source 1..20: mol_type = other DNA
acatttagggcggtcaagag

SEQ ID NO: 45 - DNA, 19 bp, synthetic construct
  misc_feature 1..19: note = Probe
  source 1..19: mol_type = other DNA
atgaagtgatccgggccat

SEQ ID NO: 46 - DNA, 21 bp, synthetic construct
  misc_feature 1..21: note = Primer
  source 1..21: mol_type = other DNA
ccgtactgcatagggatgaaa

SEQ ID NO: 47 - DNA, 21 bp, synthetic construct
  misc_feature 1..21: note = Primer
  source 1..21: mol_type = other DNA
taaggcaaaggatgggatcaa

SEQ ID NO: 48 - DNA, 21 bp, synthetic construct
  misc_feature 1..21: note = Probe
  source 1..21: mol_type = other DNA
ttgctgacgaggttgtggtag

SEQ ID NO: 49 - DNA, 300 bp, Methylobacterium sp.
  source 1..300: mol_type = genomic DNA
ggaaatcggcttcaagtacgacgtcacgccggccatgcaggtcacgggtgcactgttcaatctcgagcgcgacaaccagccgttcccctcgaacgtggagtccggcctcgtccttggcgcaggtcagacacgcacccagggcgcggaaatcggcctggccggctatctaaccgattggtggcaggtctttggcggctacgcttataccgaggcacgcgtactctcgccactggaagacgatggagacgtgatcgcagcaggtaatctcgtcggcaacgttccgctaaatactttcagtct

SEQ ID NO: 50 - DNA, 300 bp, Methylobacterium sp.
  source 1..300: mol_type = genomic DNA
cggcctggccggctatctaaccgattggtggcaggtctttggcggctacgcttataccgaggcacgcgtactctcgccactggaagacgatggagacgtgatcgcagcaggtaatctcgtcggcaacgttccgctaaatactttcagtctgttcaacaagttcgatatcaacgagaatttctccgttgctctgggctattactatcaggatgccagctttgcctcctcagacaatgcagtgcgtttgccaagttattcgcggttcgatggcgggttgttctatcgattcgacgagttgac

SEQ ID NO: 51 - DNA, 300 bp, Methylobacterium sp.
  source 1..300: mol_type = genomic DNA
acgttccgctaaatactttcagtctgttcaacaagttcgatatcaacgagaatttctccgttgctctgggctattactatcaggatgccagctttgcctcctcagacaatgcagtgcgtttgccaagttattcgcggttcgatggcgggttgttctatcgattcgacgagttgacacgcgttcagcttagcgtcgagaacattttcgacaggcgttacatcatcaactccaacaacaacaacaacctcacgcctggcgcgccgagaacagtccgcgtgcaattgatcgctcggttctaaa

SEQ ID NO: 52 - DNA, 20 bp, synthetic construct
  misc_feature 1..20: note = Primer
  source 1..20: mol_type = other DNA
tttggcggctacgcttatac

SEQ ID NO: 53 - DNA, 20 bp, synthetic construct
  misc_feature 1..20: note = Primer
  source 1..20: mol_type = other DNA
aacgttgccgacgagattac

SEQ ID NO: 54 - DNA, 22 bp, synthetic construct
  misc_feature 1..22: note = Probe
  source 1..22: mol_type = other DNA
agacgatggagacgtgatcgca

SEQ ID NO: 55 - DNA, 20 bp, synthetic construct
  misc_feature 1..20: note = Primer
  source 1..20: mol_type = other DNA
ggcaacgttccgctaaatac

SEQ ID NO: 56 - DNA, 20 bp, synthetic construct
  misc_feature 1..20: note = Primer
  source 1..20: mol_type = other DNA
aaagctggcatcctgatagt

SEQ ID NO: 57 - DNA, 22 bp, synthetic construct
  misc_feature 1..22: note = Probe
  source 1..22: mol_type = other DNA
cgagaatttctccgttgctctg

SEQ ID NO: 58 - DNA, 19 bp, synthetic construct
  misc_feature 1..19: note = Primer
  source 1..19: mol_type = other DNA
cgatggcgggttgttctat

SEQ ID NO: 59 - DNA, 18 bp, synthetic construct
  misc_feature 1..18: note = Primer
  source 1..18: mol_type = other DNA
aggcgtgaggttgttgtt

SEQ ID NO: 60 - DNA, 22 bp, synthetic construct
  misc_feature 1..22: note = Probe
  source 1..22: mol_type = other DNA
aggcgttacatcatcaactcca